European Patent Specification EP 4 039 811 B1, published September 20, 2023. Title: Improved methods for processing DNA substrates. Applicant: Swift Biosciences, Inc. Application 18165783.4. The sequence listing filed with the application follows.

SEQUENCE LISTING (127 sequences)

SEQ ID NO: 1 - DNA, 58 bp, Artificial Sequence
  Synthetic oligonucleotide
aatgatacggcgaccaccgagatctacactctttccctacacgacgctcttccgatct

SEQ ID NO: 2 - DNA, 22 bp, Artificial Sequence
  Synthetic oligonucleotide
  misc_feature (22)..(22): 3' C3 spacer (IDT)
agatcggaagagcgtcgtgtag

SEQ ID NO: 3 - DNA, 58 bp, Artificial Sequence
  Synthetic oligonucleotide
  misc_feature (1)..(1): 5' Phosphorylation (IDT)
  misc_feature (58)..(58): 3' C3 spacer (IDT)
agatcggaagagcgtcgtgtagggaaagagtgtagatctcggtggtcgccgtatcatt

SEQ ID NO: 4 - DNA, 19 bp, Artificial Sequence
  Synthetic oligonucleotide
  misc_feature (19)..(19): 3'- Dideoxythymidine  (TriLink)
acacgacgctcttccgatc

SEQ ID NO: 5 - DNA, 20 bp, Artificial Sequence
  Synthetic oligonucleotide
  misc_feature (20)..(20): 3' Phosphorylation (IDT)
acacgacgctcttccgatct

SEQ ID NO: 6 - DNA, 24 bp, Artificial Sequence
  Synthetic oligonucleotide
  misc_feature (1)..(1): 5' Phosphorylation (IDT)
tgtacctcacttctcatcactgct

SEQ ID NO: 7 - DNA, 24 bp, Artificial Sequence
  Synthetic oligonucleotide
agcagtgatgagaagtgaggtaca

SEQ ID NO: 8 - DNA, 24 bp, Artificial Sequence
  Synthetic oligonucleotide
  misc_feature (1)..(1): 5' Phosphorylation (IDT)
tgtacctcacttctcatcactgct

SEQ ID NO: 9 - DNA, 24 bp, Artificial Sequence
  Synthetic oligonucleotide
  misc_feature (1)..(1): 5' 6-carboxyfluorescein (IDT)
agcagtgatgagaagtgaggtaca

SEQ ID NO: 10 - DNA, 24 bp, Artificial Sequence
  Synthetic oligonucleotide
tgtacctcacttctcatcactgct

SEQ ID NO: 11 - DNA, 34 bp, Artificial Sequence
  Synthetic oligonucleotide
gtgactggagttcagacgtgtgctcttccgatct

SEQ ID NO: 12 - DNA, 34 bp, Artificial Sequence
  Synthetic oligonucleotide
  misc_feature (34)..(34): 3' 6-carboxyfluorescein (IDT)
tgtacctcacttctcatcactgctgtcatccgat

SEQ ID NO: 13 - DNA, 46 bp, Artificial Sequence
  Synthetic oligonucleotide
  misc_feature (46)..(46): 3' C3 spacer (IDT)
agcagtgatgagaagtgaggtacaagatcggaagagcgtcgtgtag

SEQ ID NO: 14 - DNA, 33 bp, Artificial Sequence
  Synthetic oligonucleotide
gactggagttcagacgtgtgctcttccgatctt

SEQ ID NO: 15 - DNA, 65 bp, Artificial Sequence
  Synthetic oligonucleotide
caagcagaagacggcatacgagatcgtgatgtgactggagttcagacgtgtgctcttccgatctt

SEQ ID NO: 16 - DNA, 65 bp, Artificial Sequence
  Synthetic oligonucleotide
  misc_feature (1)..(1): 5' C3 spacer (IDT)
  misc_feature (1)..(1): Phosphorothioated base
  misc_feature (2)..(2): Phosphorothioated base
  misc_feature (65)..(65): n is a, c, g, or t
caagcagaagacggcatacgagatcgtgatgtgactggagttcagacgtgtgctcttccgatctn

SEQ ID NO: 17 - DNA, 64 bp, Artificial Sequence
  Synthetic oligonucleotide
  misc_feature (1)..(1): 5' Phosphorylation (IDT)
  misc_feature (62)..(62): Phosphorothioated base
  misc_feature (63)..(63): Phosphorothioated base
  misc_feature (64)..(64): 3' C3 spacer (IDT)
agatcggaagagcacacgtctgaactccagtcacatcacgatctcgtatgccgtcttctgcttg

SEQ ID NO: 18 - DNA, 20 bp, Artificial Sequence
  Synthetic oligonucleotide
  misc_feature (20)..(20): 2', 3'- Dideoxythymidine  (TriLink)
agacgugugcucutccgatc

SEQ ID NO: 19 - DNA, 58 bp, Artificial Sequence; identical to SEQ ID NO: 1
  Synthetic oligonucleotide
  misc_feature (1)..(1): 5' C3 spacer (IDT)
  misc_feature (1)..(1): Phosphorothioated base
  misc_feature (2)..(2): Phosphorothioated base

SEQ ID NO: 20 - DNA, 59 bp, Artificial Sequence
  Synthetic oligonucleotide
  misc_feature (1)..(1): 5' C3 spacer (IDT)
  misc_feature (1)..(1): Phosphorothioated base
  misc_feature (2)..(2): Phosphorothioated base
  misc_feature (59)..(59): n is a, c, g, or t
aatgatacggcgaccaccgagatctacactctttccctacacgacgctcttccgatctn

SEQ ID NO: 21 - DNA, 64 bp, Artificial Sequence
  Synthetic oligonucleotide
  misc_feature (1)..(1): 5' Phosphorylation (IDT)
  misc_feature (62)..(62): Phosphorothioated base
  misc_feature (63)..(63): Phosphorothioated base
  misc_feature (64)..(64): 3' C3 spacer (IDT)
agatcggaagagcacacgtctgaactccagtcacgccaatatctcgtatgccgtcttctgcttg

SEQ ID NO: 22 - skipped

SEQ ID NO: 23 - DNA, 42 bp, Artificial Sequence
  Synthetic oligonucleotide
  misc_feature (40)..(40): Phosphorothioated DNA bases (IDT)
  misc_feature (41)..(41): Phosphorothioated DNA bases (IDT)
tcagacgtgtgctcttccgatctcctgcccttccaatggatc

SEQ ID NO: 24 - DNA, 41 bp, Artificial Sequence
  Synthetic oligonucleotide
  misc_feature (39)..(39): Phosphorothioated DNA bases (IDT)
  misc_feature (40)..(40): Phosphorothioated DNA bases (IDT)
tcagacgtgtgctcttccgatctcccctagcagagacctgt

SEQ ID NO: 25 - DNA, 42 bp, Artificial Sequence
  Synthetic oligonucleotide
  misc_feature (40)..(40): Phosphorothioated DNA bases (IDT)
  misc_feature (41)..(41): Phosphorothioated DNA bases (IDT)
tcagacgtgtgctcttccgatctgcccaacccttgtccttac

SEQ ID NO: 26 - DNA, 44 bp, Artificial Sequence
  Synthetic oligonucleotide
  misc_feature (42)..(42): Phosphorothioated DNA bases (IDT)
  misc_feature (43)..(43): Phosphorothioated DNA bases (IDT)
tcagacgtgtgctcttccgatctctgactgctcttttcacccat

SEQ ID NO: 27 - DNA, 43 bp, Artificial Sequence
  Synthetic oligonucleotide
  misc_feature (41)..(41): Phosphorothioated DNA bases (IDT)
  misc_feature (42)..(42): Phosphorothioated DNA bases (IDT)
tcagacgtgtgctcttccgatctgagcagcctctggcattctg

SEQ ID NO: 28 - DNA, 44 bp, Artificial Sequence
  Synthetic oligonucleotide
  misc_feature (42)..(42): Phosphorothioated DNA bases (IDT)
  misc_feature (43)..(43): Phosphorothioated DNA bases (IDT)
tcagacgtgtgctcttccgatcttgaagacccaggtccagatga

SEQ ID NO: 29 - DNA, 44 bp, Artificial Sequence
  Synthetic oligonucleotide
  misc_feature (42)..(42): Phosphorothioated DNA bases (IDT)
  misc_feature (43)..(43): Phosphorothioated DNA bases (IDT)
tcagacgtgtgctcttccgatctgctgccctggtaggttttctg

SEQ ID NO: 30 - DNA, 43 bp, Artificial Sequence
  Synthetic oligonucleotide
  misc_feature (41)..(41): Phosphorothioated DNA bases (IDT)
  misc_feature (42)..(42): Phosphorothioated DNA bases (IDT)
tcagacgtgtgctcttccgatctctggcccctgtcatcttctg

SEQ ID NO: 31 - DNA, 44 bp, Artificial Sequence
  Synthetic oligonucleotide
  misc_feature (42)..(42): Phosphorothioated DNA bases (IDT)
  misc_feature (43)..(43): Phosphorothioated DNA bases (IDT)
tcagacgtgtgctcttccgatctcaggcattgaagtctcatgga

SEQ ID NO: 32 - DNA, 42 bp, Artificial Sequence
  Synthetic oligonucleotide
  misc_feature (40)..(40): Phosphorothioated DNA bases (IDT)
  misc_feature (41)..(41): Phosphorothioated DNA bases (IDT)
tcagacgtgtgctcttccgatcttcctccctgcttctgtctc

SEQ ID NO: 33 - DNA, 44 bp, Artificial Sequence
  Synthetic oligonucleotide
  misc_feature (42)..(42): Phosphorothioated DNA bases (IDT)
  misc_feature (43)..(43): Phosphorothioated DNA bases (IDT)
tcagacgtgtgctcttccgatctctgtcagtggggaacaagaag

SEQ ID NO: 34 - DNA, 43 bp, Artificial Sequence
  Synthetic oligonucleotide
  misc_feature (41)..(41): Phosphorothioated DNA bases (IDT)
  misc_feature (42)..(42): Phosphorothioated DNA bases (IDT)
tcagacgtgtgctcttccgatctgtgctgtgactgcttgtaga

SEQ ID NO: 35 - DNA, 46 bp, Artificial Sequence
  Synthetic oligonucleotide
  misc_feature (44)..(44): Phosphorothioated DNA bases (IDT)
  misc_feature (45)..(45): Phosphorothioated DNA bases (IDT)
tcagacgtgtgctcttccgatctctctgtctccttcctcttcctac

SEQ ID NO: 36 - DNA, 42 bp, Artificial Sequence
  Synthetic oligonucleotide
  misc_feature (40)..(40): Phosphorothioated DNA bases (IDT)
  misc_feature (41)..(41): Phosphorothioated DNA bases (IDT)
tcagacgtgtgctcttccgatctctgtgcagctgtgggttga

SEQ ID NO: 37 - DNA, 43 bp, Artificial Sequence
  Synthetic oligonucleotide
  misc_feature (41)..(41): Phosphorothioated DNA bases (IDT)
  misc_feature (42)..(42): Phosphorothioated DNA bases (IDT)
tcagacgtgtgctcttccgatctgctcaccatcgctatctgag

SEQ ID NO: 38 - DNA, 42 bp, Artificial Sequence
  Synthetic oligonucleotide
  misc_feature (40)..(40): Phosphorothioated DNA bases (IDT)
  misc_feature (41)..(41): Phosphorothioated DNA bases (IDT)
tcagacgtgtgctcttccgatctcatgacggaggttgtgagg

SEQ ID NO: 39 - DNA, 45 bp, Artificial Sequence
  Synthetic oligonucleotide
  misc_feature (43)..(43): Phosphorothioated DNA bases (IDT)
  misc_feature (44)..(44): Phosphorothioated DNA bases (IDT)
tcagacgtgtgctcttccgatctagcaatcagtgaggaatcagag

SEQ ID NO: 40 - DNA, 40 bp, Artificial Sequence
  Synthetic oligonucleotide
  misc_feature (38)..(38): Phosphorothioated DNA bases (IDT)
  misc_feature (39)..(39): Phosphorothioated DNA bases (IDT)
tcagacgtgtgctcttccgatctagctggggctggagaga

SEQ ID NO: 41 - DNA, 46 bp, Artificial Sequence
  Synthetic oligonucleotide
  misc_feature (44)..(44): Phosphorothioated DNA bases (IDT)
  misc_feature (45)..(45): Phosphorothioated DNA bases (IDT)
tcagacgtgtgctcttccgatctgtcatccaaatactccacacgca

SEQ ID NO: 42 - DNA, 44 bp, Artificial Sequence
  Synthetic oligonucleotide
  misc_feature (42)..(42): Phosphorothioated DNA bases (IDT)
  misc_feature (43)..(43): Phosphorothioated DNA bases (IDT)
tcagacgtgtgctcttccgatctgcatcttatccgagtggaagg

SEQ ID NO: 43 - DNA, 44 bp, Artificial Sequence
  Synthetic oligonucleotide
  misc_feature (42)..(42): Phosphorothioated DNA bases (IDT)
  misc_feature (43)..(43): Phosphorothioated DNA bases (IDT)
tcagacgtgtgctcttccgatctcactgacaaccacccttaacc

SEQ ID NO: 44 - DNA, 46 bp, Artificial Sequence
  Synthetic oligonucleotide
  misc_feature (44)..(44): Phosphorothioated DNA bases (IDT)
  misc_feature (45)..(45): Phosphorothioated DNA bases (IDT)
tcagacgtgtgctcttccgatctcaggtaggacctgatttccttac

SEQ ID NO: 45 - DNA, 44 bp, Artificial Sequence
  Synthetic oligonucleotide
  misc_feature (42)..(42): Phosphorothioated DNA bases (IDT)
  misc_feature (43)..(43): Phosphorothioated DNA bases (IDT)
tcagacgtgtgctcttccgatctttcttgcggagattctcttcc

SEQ ID NO: 46 - DNA, 43 bp, Artificial Sequence
  Synthetic oligonucleotide
  misc_feature (41)..(41): Phosphorothioated DNA bases (IDT)
  misc_feature (42)..(42): Phosphorothioated DNA bases (IDT)
tcagacgtgtgctcttccgatcttgggacggaacagctttgag

SEQ ID NO: 47 - DNA, 41 bp, Artificial Sequence
  Synthetic oligonucleotide
  misc_feature (39)..(39): Phosphorothioated DNA bases (IDT)
  misc_feature (40)..(40): Phosphorothioated DNA bases (IDT)
tcagacgtgtgctcttccgatctccaccgcttcttgtcctg

SEQ ID NO: 48 - DNA, 42 bp, Artificial Sequence
  Synthetic oligonucleotide
  misc_feature (40)..(40): Phosphorothioated DNA bases (IDT)
  misc_feature (41)..(41): Phosphorothioated DNA bases (IDT)
tcagacgtgtgctcttccgatctgggtgcagttatgcctcag

SEQ ID NO: 49 - DNA, 45 bp, Artificial Sequence
  Synthetic oligonucleotide
  misc_feature (43)..(43): Phosphorothioated DNA bases (IDT)
  misc_feature (44)..(44): Phosphorothioated DNA bases (IDT)
tcagacgtgtgctcttccgatctagacttagtacctgaagggtga

SEQ ID NO: 50 - DNA, 43 bp, Artificial Sequence
  Synthetic oligonucleotide
  misc_feature (41)..(41): Phosphorothioated DNA bases (IDT)
  misc_feature (42)..(42): Phosphorothioated DNA bases (IDT)
tcagacgtgtgctcttccgatcttagcactgcccaacaacacc

SEQ ID NO: 51 - DNA, 46 bp, Artificial Sequence
  Synthetic oligonucleotide
  misc_feature (44)..(44): Phosphorothioated DNA bases (IDT)
  misc_feature (45)..(45): Phosphorothioated DNA bases (IDT)
tcagacgtgtgctcttccgatctcggcattttgagtgttagactgg

SEQ ID NO: 52 - DNA, 46 bp, Artificial Sequence
  Synthetic oligonucleotide
  misc_feature (44)..(44): Phosphorothioated DNA bases (IDT)
  misc_feature (45)..(45): Phosphorothioated DNA bases (IDT)
tcagacgtgtgctcttccgatctcctggttgtagctaactaacttc

SEQ ID NO: 53 - DNA, 46 bp, Artificial Sequence
  Synthetic oligonucleotide
  misc_feature (44)..(44): Phosphorothioated DNA bases (IDT)
  misc_feature (45)..(45): Phosphorothioated DNA bases (IDT)
tcagacgtgtgctcttccgatctaccatcgtaagtcaagtagcatc

SEQ ID NO: 54 - DNA, 45 bp, Artificial Sequence
  Synthetic oligonucleotide
  misc_feature (43)..(43): Phosphorothioated DNA bases (IDT)
  misc_feature (44)..(44): Phosphorothioated DNA bases (IDT)
tcagacgtgtgctcttccgatctatggttctatgactttgcctga

SEQ ID NO: 55 - DNA, 44 bp, Artificial Sequence
  Synthetic oligonucleotide
  misc_feature (42)..(42): Phosphorothioated DNA bases (IDT)
  misc_feature (43)..(43): Phosphorothioated DNA bases (IDT)
tcagacgtgtgctcttccgatctagcaggctaggctaagctatg

SEQ ID NO: 56 - DNA, 52 bp, Artificial Sequence
  Synthetic oligonucleotide
  misc_feature (50)..(50): Phosphorothioated DNA bases (IDT)
  misc_feature (51)..(51): Phosphorothioated DNA bases (IDT)
tcagacgtgtgctcttccgatctcctgctgaaaatgactgaatataaacttg

SEQ ID NO: 57 - DNA, 44 bp, Artificial Sequence
  Synthetic oligonucleotide
  misc_feature (42)..(42): Phosphorothioated DNA bases (IDT)
  misc_feature (43)..(43): Phosphorothioated DNA bases (IDT)
tcagacgtgtgctcttccgatctggtcctgcaccagtaatatgc

SEQ ID NO: 58 - DNA, 47 bp, Artificial Sequence
  Synthetic oligonucleotide
  misc_feature (45)..(45): Phosphorothioated DNA bases (IDT)
  misc_feature (46)..(46): Phosphorothioated DNA bases (IDT)
tcagacgtgtgctcttccgatcttgcttgctctgataggaaaatgag

SEQ ID NO: 59 - DNA, 47 bp, Artificial Sequence
  Synthetic oligonucleotide
  misc_feature (45)..(45): Phosphorothioated DNA bases (IDT)
  misc_feature (46)..(46): Phosphorothioated DNA bases (IDT)
tcagacgtgtgctcttccgatctggatccagacaactgttcaaactg

SEQ ID NO: 60 - DNA, 43 bp, Artificial Sequence
  Synthetic oligonucleotide
  misc_feature (41)..(41): Phosphorothioated DNA bases (IDT)
  misc_feature (42)..(42): Phosphorothioated DNA bases (IDT)
tcagacgtgtgctcttccgatctccagaaactgcctcttgacc

SEQ ID NO: 61 - DNA, 43 bp, Artificial Sequence
  Synthetic oligonucleotide
  misc_feature (41)..(41): Phosphorothioated DNA bases (IDT)
  misc_feature (42)..(42): Phosphorothioated DNA bases (IDT)
tcagacgtgtgctcttccgatctgatgtaagggacaagcagcc

SEQ ID NO: 62 - DNA, 44 bp, Artificial Sequence
  Synthetic oligonucleotide
  misc_feature (42)..(42): Phosphorothioated DNA bases (IDT)
  misc_feature (43)..(43): Phosphorothioated DNA bases (IDT)
tcagacgtgtgctcttccgatctgaaccaatggatcgatctgcc

SEQ ID NO: 63 - DNA, 44 bp, Artificial Sequence
  Synthetic oligonucleotide
  misc_feature (42)..(42): Phosphorothioated DNA bases (IDT)
  misc_feature (43)..(43): Phosphorothioated DNA bases (IDT)
tcagacgtgtgctcttccgatctggggaactgatgtgacttacc

SEQ ID NO: 64 - DNA, 43 bp, Artificial Sequence
  Synthetic oligonucleotide
  misc_feature (41)..(41): Phosphorothioated DNA bases (IDT)
  misc_feature (42)..(42): Phosphorothioated DNA bases (IDT)
tcagacgtgtgctcttccgatctctgagcaagaggctttggag

SEQ ID NO: 65 - DNA, 43 bp, Artificial Sequence
  Synthetic oligonucleotide
  misc_feature (41)..(41): Phosphorothioated DNA bases (IDT)
  misc_feature (42)..(42): Phosphorothioated DNA bases (IDT)
tcagacgtgtgctcttccgatctaacagtgcagtgtggaatcc

SEQ ID NO: 66 - DNA, 47 bp, Artificial Sequence
  Synthetic oligonucleotide
  misc_feature (45)..(45): Phosphorothioated DNA bases (IDT)
  misc_feature (46)..(46): Phosphorothioated DNA bases (IDT)
tcagacgtgtgctcttccgatctccacagaaacccatgtatgaagta

SEQ ID NO: 67 - DNA, 45 bp, Artificial Sequence
  Synthetic oligonucleotide
  misc_feature (43)..(43): Phosphorothioated DNA bases (IDT)
  misc_feature (44)..(44): Phosphorothioated DNA bases (IDT)
tcagacgtgtgctcttccgatctgtacccaaaaaggtgacatgga

SEQ ID NO: 68 - DNA, 49 bp, Artificial Sequence
  Synthetic oligonucleotide
  misc_feature (47)..(47): Phosphorothioated DNA bases (IDT)
  misc_feature (48)..(48): Phosphorothioated DNA bases (IDT)
tcagacgtgtgctcttccgatcttttcagtgttacttacctgtcttgtc

SEQ ID NO: 69 - DNA, 48 bp, Artificial Sequence
  Synthetic oligonucleotide
  misc_feature (46)..(46): Phosphorothioated DNA bases (IDT)
  misc_feature (47)..(47): Phosphorothioated DNA bases (IDT)
tcagacgtgtgctcttccgatctggactctgaagatgtacctatggtc

SEQ ID NO: 70 - DNA, 43 bp, Artificial Sequence
  Synthetic oligonucleotide
  misc_feature (41)..(41): Phosphorothioated DNA bases (IDT)
  misc_feature (42)..(42): Phosphorothioated DNA bases (IDT)
tcagacgtgtgctcttccgatctctcaccatgtcctgactgtg

SEQ ID NO: 71 - DNA, 40 bp, Artificial Sequence
  Synthetic oligonucleotide
  misc_feature (38)..(38): Phosphorothioated DNA bases (IDT)
  misc_feature (39)..(39): Phosphorothioated DNA bases (IDT)
tcagacgtgtgctcttccgatctgtggcactctggaagca

SEQ ID NO: 72 - DNA, 45 bp, Artificial Sequence
  Synthetic oligonucleotide
  misc_feature (43)..(43): Phosphorothioated DNA bases (IDT)
  misc_feature (44)..(44): Phosphorothioated DNA bases (IDT)
tcagacgtgtgctcttccgatctgttactgaaagctcagggatag

SEQ ID NO: 73 - DNA, 45 bp, Artificial Sequence
  Synthetic oligonucleotide
  misc_feature (43)..(43): Phosphorothioated DNA bases (IDT)
  misc_feature (44)..(44): Phosphorothioated DNA bases (IDT)
tcagacgtgtgctcttccgatctccacacttacacatcactttgc

SEQ ID NO: 74 - DNA, 46 bp, Artificial Sequence
  Synthetic oligonucleotide
  misc_feature (44)..(44): Phosphorothioated DNA bases (IDT)
  misc_feature (45)..(45): Phosphorothioated DNA bases (IDT)
tcagacgtgtgctcttccgatcttagtctttctttgaagcagcaag

SEQ ID NO: 75 - DNA, 46 bp, Artificial Sequence
  Synthetic oligonucleotide
  misc_feature (44)..(44): Phosphorothioated DNA bases (IDT)
  misc_feature (45)..(45): Phosphorothioated DNA bases (IDT)
tcagacgtgtgctcttccgatctctagctgtgatcctgaaactgaa

SEQ ID NO: 76 - DNA, 43 bp, Artificial Sequence
  Synthetic oligonucleotide
  misc_feature (41)..(41): Phosphorothioated DNA bases (IDT)
  misc_feature (42)..(42): Phosphorothioated DNA bases (IDT)
tcagacgtgtgctcttccgatcttcctcctgcaggattcctac

SEQ ID NO: 77 - DNA, 44 bp, Artificial Sequence
  Synthetic oligonucleotide
  misc_feature (42)..(42): Phosphorothioated DNA bases (IDT)
  misc_feature (43)..(43): Phosphorothioated DNA bases (IDT)
tcagacgtgtgctcttccgatcttggtggatgtcctcaaaagac

SEQ ID NO: 78 - DNA, 49 bp, Artificial Sequence
  Synthetic oligonucleotide
  misc_feature (47)..(47): Phosphorothioated DNA bases (IDT)
  misc_feature (48)..(48): Phosphorothioated DNA bases (IDT)
tcagacgtgtgctcttccgatctcaggattcttacagaaaacaagtggt

SEQ ID NO: 79 - DNA, 46 bp, Artificial Sequence
  Synthetic oligonucleotide
  misc_feature (44)..(44): Phosphorothioated DNA bases (IDT)
  misc_feature (45)..(45): Phosphorothioated DNA bases (IDT)
tcagacgtgtgctcttccgatcttgatggcaaatacacagaggaag

SEQ ID NO: 80 - DNA, 42 bp, Artificial Sequence
  Synthetic oligonucleotide
  misc_feature (40)..(40): Phosphorothioated DNA bases (IDT)
  misc_feature (41)..(41): Phosphorothioated DNA bases (IDT)
tcagacgtgtgctcttccgatctgacgggtagagtgtgcgtg

SEQ ID NO: 81 - DNA, 44 bp, Artificial Sequence
  Synthetic oligonucleotide
  misc_feature (42)..(42): Phosphorothioated DNA bases (IDT)
  misc_feature (43)..(43): Phosphorothioated DNA bases (IDT)
tcagacgtgtgctcttccgatctcgccacagagaagttgttgag

SEQ ID NO: 82 - DNA, 41 bp, Artificial Sequence
  Synthetic oligonucleotide
  misc_feature (39)..(39): Phosphorothioated DNA bases (IDT)
  misc_feature (40)..(40): Phosphorothioated DNA bases (IDT)
tcagacgtgtgctcttccgatctcgcactggcctcatcttg

SEQ ID NO: 83 - DNA, 45 bp, Artificial Sequence
  Synthetic oligonucleotide
  misc_feature (43)..(43): Phosphorothioated DNA bases (IDT)
  misc_feature (44)..(44): Phosphorothioated DNA bases (IDT)
tcagacgtgtgctcttccgatctcttccagtgtgatgatggtgag

SEQ ID NO: 84 - DNA, 45 bp, Artificial Sequence
  Synthetic oligonucleotide
  misc_feature (43)..(43): Phosphorothioated DNA bases (IDT)
  misc_feature (44)..(44): Phosphorothioated DNA bases (IDT)
tcagacgtgtgctcttccgatctcatgtgtaacagttcctgcatg

SEQ ID NO: 85 - DNA, 41 bp, Artificial Sequence
  Synthetic oligonucleotide
  misc_feature (39)..(39): Phosphorothioated DNA bases (IDT)
  misc_feature (40)..(40): Phosphorothioated DNA bases (IDT)
tcagacgtgtgctcttccgatctggtcagaggcaagcagag

SEQ ID NO: 86 - DNA, 43 bp, Artificial Sequence
  Synthetic oligonucleotide
  misc_feature (41)..(41): Phosphorothioated DNA bases (IDT)
  misc_feature (42)..(42): Phosphorothioated DNA bases (IDT)
tcagacgtgtgctcttccgatctttacttctccccctcctctg

SEQ ID NO: 87 - DNA, 41 bp, Artificial Sequence
  Synthetic oligonucleotide
  misc_feature (39)..(39): Phosphorothioated DNA bases (IDT)
  misc_feature (40)..(40): Phosphorothioated DNA bases (IDT)
tcagacgtgtgctcttccgatctcttcccagcctgggcatc

SEQ ID NO: 88 - DNA, 43 bp, Artificial Sequence
  Synthetic oligonucleotide
  misc_feature (41)..(41): Phosphorothioated DNA bases (IDT)
  misc_feature (42)..(42): Phosphorothioated DNA bases (IDT)
tcagacgtgtgctcttccgatctgctgaatgaggccttggaac

SEQ ID NO: 89 - DNA, 44 bp, Artificial Sequence
  Synthetic oligonucleotide
  misc_feature (42)..(42): Phosphorothioated DNA bases (IDT)
  misc_feature (43)..(43): Phosphorothioated DNA bases (IDT)
tcagacgtgtgctcttccgatctctttccaacctaggaaggcag

SEQ ID NO: 90 - DNA, 47 bp, Artificial Sequence
  Synthetic oligonucleotide
  misc_feature (45)..(45): Phosphorothioated DNA bases (IDT)
  misc_feature (46)..(46): Phosphorothioated DNA bases (IDT)
tcagacgtgtgctcttccgatctgcactgtaataatccagactgtgt

SEQ ID NO: 91 - DNA, 44 bp, Artificial Sequence
  Synthetic oligonucleotide
  misc_feature (42)..(42): Phosphorothioated DNA bases (IDT)
  misc_feature (43)..(43): Phosphorothioated DNA bases (IDT)
tcagacgtgtgctcttccgatctcatgtactggtccctcattgc

SEQ ID NO: 92 - DNA, 44 bp, Artificial Sequence
  Synthetic oligonucleotide
  misc_feature (42)..(42): Phosphorothioated DNA bases (IDT)
  misc_feature (43)..(43): Phosphorothioated DNA bases (IDT)
tcagacgtgtgctcttccgatctcctttcaggatggtggatgtg

SEQ ID NO: 93 - DNA, 41 bp, Artificial Sequence
  Synthetic oligonucleotide
  misc_feature (39)..(39): Phosphorothioated DNA bases (IDT)
  misc_feature (40)..(40): Phosphorothioated DNA bases (IDT)
tcagacgtgtgctcttccgatctcgactccaccaggacttg

SEQ ID NO: 94 - DNA, 46 bp, Artificial Sequence
  Synthetic oligonucleotide
  misc_feature (44)..(44): Phosphorothioated DNA bases (IDT)
  misc_feature (45)..(45): Phosphorothioated DNA bases (IDT)
tcagacgtgtgctcttccgatctgttaaccttgcagaatggtcgat

SEQ ID NO: 95 - DNA, 47 bp, Artificial Sequence
  Synthetic oligonucleotide
  misc_feature (45)..(45): Phosphorothioated DNA bases (IDT)
  misc_feature (46)..(46): Phosphorothioated DNA bases (IDT)
tcagacgtgtgctcttccgatctccacgagaacttgatcatattcac

SEQ ID NO: 96 - DNA, 44 bp, Artificial Sequence
  Synthetic oligonucleotide
  misc_feature (42)..(42): Phosphorothioated DNA bases (IDT)
  misc_feature (43)..(43): Phosphorothioated DNA bases (IDT)
tcagacgtgtgctcttccgatctcaacaggttcttgctggtgtg

SEQ ID NO: 97 - DNA, 47 bp, Artificial Sequence
  Synthetic oligonucleotide
  misc_feature (45)..(45): Phosphorothioated DNA bases (IDT)
  misc_feature (46)..(46): Phosphorothioated DNA bases (IDT)
tcagacgtgtgctcttccgatctatggtgggatcatattcatctaca

SEQ ID NO: 98 - DNA, 43 bp, Artificial Sequence
  Synthetic oligonucleotide
  misc_feature (41)..(41): Phosphorothioated DNA bases (IDT)
  misc_feature (42)..(42): Phosphorothioated DNA bases (IDT)
tcagacgtgtgctcttccgatctagcttgtggagcctcttaca

SEQ ID NO: 99 - DNA, 45 bp, Artificial Sequence
  Synthetic oligonucleotide
  misc_feature (43)..(43): Phosphorothioated DNA bases (IDT)
  misc_feature (44)..(44): Phosphorothioated DNA bases (IDT)
tcagacgtgtgctcttccgatctgggaccttaccttatacaccgt

SEQ ID NO: 100 - DNA, 44 bp, Artificial Sequence
  Synthetic oligonucleotide
  misc_feature (42)..(42): Phosphorothioated DNA bases (IDT)
  misc_feature (43)..(43): Phosphorothioated DNA bases (IDT)
tcagacgtgtgctcttccgatctcaccatctcacaattgccagt

SEQ ID NO: 101 - DNA, 45 bp, Artificial Sequence
  Synthetic oligonucleotide
  misc_feature (43)..(43): Phosphorothioated DNA bases (IDT)
  misc_feature (44)..(44): Phosphorothioated DNA bases (IDT)
tcagacgtgtgctcttccgatctgctttcggagatgttgcttctc

SEQ ID NO: 102 - DNA, 45 bp, Artificial Sequence
  Synthetic oligonucleotide
  misc_feature (43)..(43): Phosphorothioated DNA bases (IDT)
  misc_feature (44)..(44): Phosphorothioated DNA bases (IDT)
tcagacgtgtgctcttccgatctgatcccagaaggtgagaaagtt

SEQ ID NO: 103 - DNA, 42 bp, Artificial Sequence
  Synthetic oligonucleotide
  misc_feature (40)..(40): Phosphorothioated DNA bases (IDT)
  misc_feature (41)..(41): Phosphorothioated DNA bases (IDT)
tcagacgtgtgctcttccgatcttgaggttcagagccatgga

SEQ ID NO: 104 - DNA, 42 bp, Artificial Sequence
  Synthetic oligonucleotide
  misc_feature (40)..(40): Phosphorothioated DNA bases (IDT)
  misc_feature (41)..(41): Phosphorothioated DNA bases (IDT)
tcagacgtgtgctcttccgatctctccaggaagcctacgtga

SEQ ID NO: 105 - DNA, 42 bp, Artificial Sequence
  Synthetic oligonucleotide
  misc_feature (40)..(40): Phosphorothioated DNA bases (IDT)
  misc_feature (41)..(41): Phosphorothioated DNA bases (IDT)
tcagacgtgtgctcttccgatctggacatagtccaggaggca

SEQ ID NO: 106 - DNA, 43 bp, Artificial Sequence
  Synthetic oligonucleotide
  misc_feature (41)..(41): Phosphorothioated DNA bases (IDT)
  misc_feature (42)..(42): Phosphorothioated DNA bases (IDT)
tcagacgtgtgctcttccgatctcaccgcagcatgtcaagatc

SEQ ID NO: 107 - DNA, 44 bp, Artificial Sequence
  Synthetic oligonucleotide
  misc_feature (42)..(42): Phosphorothioated DNA bases (IDT)
  misc_feature (43)..(43): Phosphorothioated DNA bases (IDT)
tcagacgtgtgctcttccgatctgacctaaagccacctccttac

SEQ ID NO: 108 - DNA, 46 bp, Artificial Sequence
  Synthetic oligonucleotide
  misc_feature (44)..(44): Phosphorothioated DNA bases (IDT)
  misc_feature (45)..(45): Phosphorothioated DNA bases (IDT)
tcagacgtgtgctcttccgatcttccactatactgacgtctccaac

SEQ ID NO: 109 - DNA, 46 bp, Artificial Sequence
  Synthetic oligonucleotide
  misc_feature (44)..(44): Phosphorothioated DNA bases (IDT)
  misc_feature (45)..(45): Phosphorothioated DNA bases (IDT)
tcagacgtgtgctcttccgatctacacacgcaaaatactccttcag

SEQ ID NO: 110 - DNA, 44 bp, Artificial Sequence
  Synthetic oligonucleotide
  misc_feature (42)..(42): Phosphorothioated DNA bases (IDT)
  misc_feature (43)..(43): Phosphorothioated DNA bases (IDT)
tcagacgtgtgctcttccgatctctgtcctcacagagttcaagc

SEQ ID NO: 111 - DNA, 45 bp, Artificial Sequence
  Synthetic oligonucleotide
  misc_feature (43)..(43): Phosphorothioated DNA bases (IDT)
  misc_feature (44)..(44): Phosphorothioated DNA bases (IDT)
tcagacgtgtgctcttccgatctgtttttgcagatgatgggctcc

SEQ ID NO: 112 - DNA, 41 bp, Artificial Sequence
  Synthetic oligonucleotide
  misc_feature (39)..(39): Phosphorothioated DNA bases (IDT)
  misc_feature (40)..(40): Phosphorothioated DNA bases (IDT)
tcagacgtgtgctcttccgatctctggaccaagcccatcac

SEQ ID NO: 113 - DNA, 42 bp, Artificial Sequence
  Synthetic oligonucleotide
  misc_feature (40)..(40): Phosphorothioated DNA bases (IDT)
  misc_feature (41)..(41): Phosphorothioated DNA bases (IDT)
tcagacgtgtgctcttccgatcttgtggccttgtactgcaga

SEQ ID NO: 114 - DNA, 44 bp, Artificial Sequence
  Synthetic oligonucleotide
  misc_feature (42)..(42): Phosphorothioated DNA bases (IDT)
  misc_feature (43)..(43): Phosphorothioated DNA bases (IDT)
tcagacgtgtgctcttccgatctcagtgtgttcacagagacctg

SEQ ID NO: 115 - DNA, 45 bp, Artificial Sequence
  Synthetic oligonucleotide
  misc_feature (43)..(43): Phosphorothioated DNA bases (IDT)
  misc_feature (44)..(44): Phosphorothioated DNA bases (IDT)
tcagacgtgtgctcttccgatctgtaggaaatagcagcctcacat

SEQ ID NO: 116 - DNA, 46 bp, Artificial Sequence
  Synthetic oligonucleotide
  misc_feature (44)..(44): Phosphorothioated DNA bases (IDT)
  misc_feature (45)..(45): Phosphorothioated DNA bases (IDT)
tcagacgtgtgctcttccgatcttgttcctgatctccttagacaac

SEQ ID NO: 117 - DNA, 43 bp, Artificial Sequence
  Synthetic oligonucleotide
  misc_feature (41)..(41): Phosphorothioated DNA bases (IDT)
  misc_feature (42)..(42): Phosphorothioated DNA bases (IDT)
tcagacgtgtgctcttccgatctcttgctgcacttctcacacc

SEQ ID NO: 118 - DNA, 44 bp, Artificial Sequence
  Synthetic oligonucleotide
  misc_feature (42)..(42): Phosphorothioated DNA bases (IDT)
  misc_feature (43)..(43): Phosphorothioated DNA bases (IDT)
tcagacgtgtgctcttccgatcttgaaaattccagtggccatca

SEQ ID NO: 119 - DNA, 43 bp, Artificial Sequence
  Synthetic oligonucleotide
  misc_feature (41)..(41): Phosphorothioated DNA bases (IDT)
  misc_feature (42)..(42): Phosphorothioated DNA bases (IDT)
tcagacgtgtgctcttccgatctcaatgaagagagaccagagc

SEQ ID NO: 120 - DNA, 43 bp, Artificial Sequence
  Synthetic oligonucleotide
  misc_feature (41)..(41): Phosphorothioated DNA bases (IDT)
  misc_feature (42)..(42): Phosphorothioated DNA bases (IDT)
tcagacgtgtgctcttccgatctcccataccctctcagcgtac

SEQ ID NO: 121 - DNA, 42 bp, Artificial Sequence
  Synthetic oligonucleotide
  misc_feature (40)..(40): Phosphorothioated DNA bases (IDT)
  misc_feature (41)..(41): Phosphorothioated DNA bases (IDT)
tcagacgtgtgctcttccgatctgtggatgtcaggcagatgc

SEQ ID NO: 122 - DNA, 43 bp, Artificial Sequence
  Synthetic oligonucleotide
  misc_feature (41)..(41): Phosphorothioated DNA bases (IDT)
  misc_feature (42)..(42): Phosphorothioated DNA bases (IDT)
tcagacgtgtgctcttccgatctccctcccagaaggtctacat

SEQ ID NO: 123 - DNA, 46 bp, Artificial Sequence
  Synthetic oligonucleotide
  misc_feature (44)..(44): Phosphorothioated DNA bases (IDT)
  misc_feature (45)..(45): Phosphorothioated DNA bases (IDT)
tcagacgtgtgctcttccgatctttttgacatggttgggactcttg

SEQ ID NO: 124 - DNA, 23 bp, Artificial Sequence
  Synthetic oligonucleotide
  misc_feature (21)..(21): Phosphorothioated DNA bases (IDT)
  misc_feature (22)..(22): Phosphorothioated DNA bases (IDT)
tcagacgugugcucuuccgaucu

SEQ ID NO: 125 - DNA, 21 bp, Artificial Sequence
  Synthetic oligonucleotide
  misc_feature (21)..(21): 3' Phosphorylation (IDT)
gtgactggagttcagacgtgt

SEQ ID NO: 126 - DNA, 44 bp, Artificial Sequence
  Synthetic oligonucleotide
  misc_feature (44)..(44): 3' Phosphorylation (IDT)
aactccagtcactaatgcgcatctcgtatgccgtcttctgcttg

SEQ ID NO: 127 - DNA, 70 bp, Artificial Sequence
  Synthetic oligonucleotide
aatgatacggcgaccaccgagatctacacaggcgaagacactctttccctacacgacgctcttccgatct